European Patent Specification EP 3 878 953 B1, published August 12, 2026. Title: Monooxygenase mutant and use thereof. Applicant: ASYMCHEM LABORATORIES (TIANJIN) CO.,LTD. Application EP18939722.7. The sequence listing filed with the application follows.

SEQUENCE LISTING (2 sequences)

SEQ ID NO: 1 - protein, 603 aa, Rhodococcus ruber-SD1
MTTSIDREALRRKYAEERDKRIRPDGNDQYIRLDHVDGWSHDPYMPITPREPKLDHVTFAFIGGGFSGLVTAARLRESGVESVRIIDKAGDFGGVWYWNRYPGAMCDTAAMVYMPLLEETGYMPTEKYAHGPEILEHCQRIGKHYDLYDDALFHTEVTDLVWQEHDQRWRISTNRGDHFTAQFVGMGTGPLHVAQLPGIPGIESFRGKSFHTSRWDYDYTGGDALGAPMDKLADKRVAVIGTGATAVQCVPELAKYCRELYVVQRTPSAVDERGNHPIDEKWFAQIATPGWQKRWLDSFTAIWDGVLTDPSELAIEHEDLVQDGWTALGQRMRAAVGSVPIEQYSPENVQRALEEADDEQMERIRARVDEIVTDPATAAQLKAWFRQMCKRPCFHDDYLPAFNRPNTHLVDTGGKGVERITENGVVVAGVEYEVDCIVYASGFEFLGTGYTDRAGFDPTGRDGVKLSEHWAQGTRTLHGMHTYGFPNLFVLQLMQGAALGSNIPHNFVEAARVVAAIVDHVLSTGTSSVETTKEAEQAWVQLLLDHGRPLGNPECTPGYYNNEGKPAELKDRLNVGYPAGSAAFFRMMDHWLAAGSFDGLTFR

SEQ ID NO: 2 - DNA, 1812 bp, Rhodococcus ruber-SD1
atgacaaccagtatcgatcgcgaggccctgcgccgcaaatatgccgaagagcgcgataaacgcatccgcccggatggcaacgatcagtatattcgcctggatcatgttgacggttggagccatgacccttatatgccgatcaccccgcgcgagccgaaactggaccatgttacatttgcattcatcggcggcggttttagcggtctggtgaccgccgcacgtctgcgtgaaagtggcgtggagagtgttcgcatcatcgacaaagcaggcgatttcggcggcgtttggtattggaaccgttatccgggtgccatgtgcgataccgcagcaatggtgtacatgcctctgctggaagagaccggctacatgccgacagaaaaatatgctcatggtccggagattctggagcactgtcagcgcatcggcaaacactacgacctgtatgacgatgccctgttccataccgaagttaccgacctggtgtggcaggagcatgatcagcgttggcgcatcagcacaaaccgcggtgaccatttcaccgcacagttcgttggcatgggtaccggcccgctgcacgttgcacagctgccgggtattccgggtatcgagagcttccgtggtaagagcttccataccagccgctgggactatgactatacaggtggcgacgcactgggcgcacctatggacaaactggcagacaaacgcgtggcagtgattggtaccggcgcaaccgccgttcagtgcgttccggaactggccaagtactgccgcgaactgtatgtggttcagcgcaccccgagtgccgttgatgaacgcggcaaccatccgatcgatgaaaagtggttcgcccagattgccacacctggttggcagaaacgctggctggatagctttaccgcaatctgggatggtgtgctgacagatccgagcgaactggccatcgagcatgaagacctggtgcaggatggttggacagcactgggtcagcgcatgcgtgcagccgtgggtagcgttccgattgaacagtatagcccggagaacgtgcagcgtgccctggaagaggccgacgatgaacagatggaacgcattcgcgcacgtgtggatgagattgtgaccgatcctgccaccgccgcccagctgaaagcatggtttcgccagatgtgcaagcgtccgtgcttccacgatgactatctgcctgcattcaaccgcccgaatacccatctggtggacacaggtggcaaaggcgtggagcgcattaccgaaaacggtgtggtggttgcaggtgtggaatatgaggtggactgcatcgtgtacgccagtggcttcgagttcttaggcaccggttatacagaccgtgcaggtttcgatccgaccggccgtgatggcgttaaactgagcgaacattgggcccaaggcacacgtaccctgcatggcatgcatacctacggctttccgaacctgtttgtgctgcagctgatgcagggtgcagccctgggtagcaacatcccgcacaactttgttgaagccgcccgcgtggtggccgcaattgttgatcatgtgctgagcacaggcaccagtagcgttgaaaccaccaaggaagccgaacaagcctgggtgcagctgctgctggatcacggtcgccctctgggcaacccggagtgtacacctggttattacaataatgaaggcaaaccggccgaactgaaggaccgtctgaacgttggctatccggccggtagcgccgccttttttcgtatgatggaccactggctggcagccggcagttttgatggcctgacattccgctaa